European Patent Application EP 4 371 998 A1, published May 22, 2024. Title: MUTANT OF PORIN MONOMER, PROTEIN PORE, AND USE THEREOF. Applicant: QITAN TECHNOLOGY LTD., CHENGDU. The sequence listing filed with the application follows.

SEQUENCE LISTING (28 sequences)

SEQ ID NO: 1 - protein, 312 aa, Thermodesulfovibrio
MFNFIKFKFILILFLPPILFGCMAMTPNIASIRATSGPEYITSIHRDLVSLPKPENPIPVAVYKFRDQTGQYKAPGNATNFSTAVTQGATSILIKALEDSGWFLPVEREGLANLLQERKIVLQMRELYLTEEQKKQFEPLPPLLYAGIIFEGGIIGYDSNVTTGGIGAKYFGAGGSAEYRVDKVSIYLRAVSVKNGAVLKTVQTSKTVLSQMLSLGIFRFVRLNRLLEAEAGIAANEPVEMAVQEAIEKAVYDIIIEGVKTGIWKPKDTKEFEKWLSKYENELKEKTFASESISKLSKQKESKDIVKELFKY

SEQ ID NO: 2 - DNA, 939 bp, Thermodesulfovibrio
atgttcaacttcatcaagttcaagttcatcctgatcctgttcctgccgccgatcctgtttggttgcatggcgatgaccccgaacattgcgagcatccgtgcgaccagcggtccggagtacattaccagcatccaccgtgacctggtgagcctgccgaaaccggaaaatccgatcccggtggcggtttacaaattccgtgatcagaccggtcaatataaggcgccgggcaacgcgaccaattttagcaccgcggttacccagggtgcgaccagcattctgatcaaagcgctggaggacagcggttggttcctgccggtggagcgtgaaggcctggcgaacctgctgcaggagcgcaagatcgttctgcaaatgcgtgaactgtacctgaccgaggaacagaagaaacaatttgagccgctgccgccgctgctgtatgcgggtatcatttttgaaggtggcatcattggctatgacagcaacgtgaccaccggtggcattggtgcgaaatattttggtgcgggtggcagcgcggagtaccgtgtggataaagttagcatctatctgcgtgctgtgagcgttaagaatggtgcggtgctgaaaaccgttcagaccagcaagaccgtgctgagccaaatgctgagcctgggtattttccgttttgttcgcctgaaccgtctgctggaggcggaagcgggtattgcggcgaatgagccggtggaaatggcggttcaggaagcgatcgaaaaagcggtgtacgacatcattatcgaaggtgttaagaccggcatctggaagccgaaagataccaaggagttcgaaaaatggctgagcaagtatgagaacgaactgaaggagaaaacctttgcgagcgaaagcattagcaagctgagcaagcaaaaagagagcaaagatatcgttaaggaactgttcaaatattaa

SEQ ID NO: 3 - DNA, 10 bp, Artificial Sequence
  part of BS7-4C3-SE1
tttttttttt

SEQ ID NO: 4 - DNA, 28 bp, Artificial Sequence
  part of BS7-4C3-SE1
aatgtacttcgttcagttacgtattgct

SEQ ID NO: 5 - DNA, 42 bp, Artificial Sequence
  part of BS7-4C3-SE1
gcaatacgtaactgaacgaagttcactatcgcattctcatga

SEQ ID NO: 6 - DNA, 20 bp, Artificial Sequence
  part of BS7-4C3-SE1
tcatgagaatgcgatagtga

SEQ ID NO: 7 - DNA, 89 bp, Artificial Sequence
  part of BS7-4C3-SE1
aaaaaaaaaaaaaaaaaaaaaaaaaaaaaaaaaaaaaaaaaagcaatacgtaactgaacgaagtacattaaaaaaaaaaaaaaaaaaaa

SEQ ID NO: 8 - DNA, 24 bp, Artificial Sequence
  part of BS7-4C3-SE1
atcctttttttttttttttttttt

SEQ ID NO: 9 - DNA, 48 bp, Artificial Sequence
  part of BS7-4C3-SE1
aatgtacttcgttcagttacgtattgcttttttttttttttttttttt

SEQ ID NO: 10 - DNA, 20 bp, Artificial Sequence
  part of BS7-4C3-SE1
tttttttttttttttttttt

SEQ ID NO: 11 - DNA, 10 bp, Artificial Sequence
  part of BS7-4C3-PLT
tttttttttt

SEQ ID NO: 12 - DNA, 28 bp, Artificial Sequence
  part of BS7-4C3-PLT
aatgtacttcgttcagttacgtattgct

SEQ ID NO: 13 - DNA, 42 bp, Artificial Sequence; identical to SEQ ID NO: 5
  part of BS7-4C3-PLT

SEQ ID NO: 14 - DNA, 20 bp, Artificial Sequence
  part of BS7-4C3-PLT
tcatgagaatgcgatagtga

SEQ ID NO: 15 - DNA, 28 bp, Artificial Sequence
  part of BS7-4C3-PLT
aaaaaaaaaaaaaaaaaaaaaaaaaaaa

SEQ ID NO: 16 - DNA, 12 bp, Artificial Sequence
  part of BS7-4C3-PLT
aaaaaaaaaaaa

SEQ ID NO: 17 - DNA, 132 bp, Artificial Sequence
  part of BS7-4C3-PLT
aaaaaaaaaaaaaatctctgaatctctgaatctctgaatctctaaaaaaaaaaaagaaaaaaaaaaaacaaaaaaaaaaaataaaaaaaaaaaaagcaatacgtaactgaacgaagtacattaaaaaaaaaa

SEQ ID NO: 18 - DNA, 42 bp, Artificial Sequence
  part of BS7-4C3-PLT
atccttttttttttaatgtacttcgttcagttacgtattgct

SEQ ID NO: 19 - DNA, 94 bp, Artificial Sequence
  part of BS7-4C3-PLT
ttttttttttttattttttttttttgttttttttttttcttttttttttttagagattcagagattcagagattcagagatttttttttttttt

SEQ ID NO: 20 - DNA, 12 bp, Artificial Sequence
  part of BS7-4C3-PLT
tttttttttttt

SEQ ID NO: 21 - DNA, 28 bp, Artificial Sequence
  part of BS7-4C3-PLT
tttttttttttttttttttttttttttt

SEQ ID NO: 22 - protein, 441 aa, Artificial Sequence
  helicase
MITIDQLTEGQFDSLQRAKVLIQEATKNDGNWNHRTKHLTINGPAGTGKTTMMKFLVSWLRDEGITGVALAAPTHAAKKVLANAVGEEVSTIHSILKINPTTYECKQFFEQSAPPDLSKIRILICEECSFYDIKLFEILMNSIQPWTIIIGIGDRAQLRPADDKGISRFFTDQRFEQTYLTEIKRSNMPIIEVATEIRNGGWIRENIIDDLGVKQDKSVSEFMTNYFKVVKSIDDLYETRMYAYTNNSVDTLNKIIRKKLYETEQDFIVGEPIVMQEPLIRDINYEGKRFQEIVFNNGEYLEVSEIKPMESVLKCRNIDYQLVLHYYQLKVKSIDTGESGLINTISDKNELNKFYMFLGKVCQDYKSGTIKAFWDDFWKIKNNYHRVKPLPVSTIHKGQGSTVDNSFLYTPCITKYAEPDLASQLLYVGVTRARHNVNFVG

SEQ ID NO: 23 - DNA, 1326 bp, Artificial Sequence
  helicase
atgatcaccatcgaccagctgaccgaaggtcagttcgactctctgcagcgtgctaaagttctgatccaggaagctaccaaaaacgacggtaactggaaccaccgtaccaaacacctgaccatcaacggtccggctggtaccggtaaaaccaccatgatgaaattcctggtttcttggctgcgtgacgaaggtatcaccggtgttgctctggctgctccgacccacgctgctaaaaaagttctggctaacgctgttggtgaagaagtttctaccatccactctatcctgaaaatcaacccgaccacctacgaatgcaaacagttcttcgaacagtctgctccgccggacctgtctaaaatccgtatcctgatctgcgaagaatgctctttctacgacatcaaactgttcgaaatcctgatgaactctatccagccgtggaccatcatcatcggtatcggtgaccgtgctcagctgcgtccggctgacgacaaaggtatctctcgtttcttcaccgaccagcgtttcgaacagacctacctgaccgaaatcaaacgttctaacatgccgatcatcgaagttgctaccgaaatccgtaacggtggttggattcgtgaaaacatcatcgacgacctgggtgttaaacaggacaaatctgtttctgaatttatgaccaactacttcaaagttgttaaatctatcgacgacctgtacgaaacccgtatgtacgcttacaccaacaactctgttgacaccctgaacaaaatcatccgtaaaaaactgtacgaaaccgaacaggacttcatcgttggtgaaccgatcgttatgcaggaaccgctgatccgtgacatcaactacgaaggtaaacgtttccaggaaatcgttttcaacaacggtgaatacctggaagtttctgaaatcaaaccgatggaatctgttctgaaatgccgtaacatcgactaccagctggttctgcactactaccagctgaaagttaaatctatcgacaccggtgaatctggtctgatcaacaccatctctgacaaaaacgaactgaacaaattctacatgttcctgggtaaagtttgccaggactacaaatctggtaccatcaaagcgttctgggacgacttctggaaaatcaaaaacaactaccaccgtgttaaaccgctgccggtttctaccatccacaaaggtcagggttctaccgttgacaactctttcctgtacaccccgtgcatcaccaaatacgctgaaccggacctggcttctcagctgctgtacgttggtgttacccgtgctcgtcacaacgttaacttcgttggttaa

SEQ ID NO: 24 - protein, 310 aa, Artificial Sequence
  mutant 1
MFNFIKFKFILILFLPPILFGCMAMTPNIASIRATSGPEYITSIHRDLVSLPKPENPIPVAVYKFRDQTGQYKPYPANASTAVTQGATSILIKALEDSGWFLPVEREGLANLLQERKIVLQMRELYLTEEQKKQFEPLPPLLYAGIIFEGGIIGYDSNVTTGGIGAKYFGAGGSAEYRVDKVSIYLRAVSVKNGAVLKTVQTSKTVLSQMLSLGIFRFVRLNRLLEAEAGIAANEPVEMAVQEAIEKAVYDIIIEGVKTGIWKPKDTKEFEKWLSKYENELKEKTFASESISKLSKQKESKDIVKELFKY

SEQ ID NO: 25 - DNA, 933 bp, Artificial Sequence
  mutant 1
atgtttaattttattaagtttaaattcatacttatcttgttcctgccgcctattctctttggctgcatggcaatgaccccgaatattgcgtccattcgtgctactagtggtccggagtacattacctcgattcatcgtgacctggttagcctgccgaaaccggaaaacccgattccggtagccgtttataaattccgcgaccagaccggtcagtataaaccgtacccggctaatgcttcgaccgcagtgacccagggtgcgacctctatcctgatcaaagcactagaagatagcggttggtttctcccagtggaacgcgagggcctggcgaatctgttgcaagagcgcaaaatcgtgctgcagatgcgtgaactgtacttgaccgaagagcagaagaaacaatttgagccgctcccaccgttgttgtacgcaggcatcatcttcgaaggtggcattatcggctatgatagcaacgtgaccactggtggtatcggtgctaagtattttggcgcgggtggtagcgcggaataccgtgttgataaagtttccatatatctgagagcggtgagcgttaagaacggtgcggttcttaagaccgttcaaacctcgaagacggtcctgtcccagatgctgagcctgggcatcttccgctttgttcgtctgaaccgtctgttagaggccgaagctggcatcgctgccaatgaaccggtcgaaatggcggtgcaagaggcgattgaaaaagcggtctacgacattattatcgagggcgttaagacgggtatttggaaaccgaaagataccaaagagttcgaaaaatggctgagcaagtacgagaacgagctgaaagagaagacgtttgcgtccgaatctatcagcaagctgtcaaagcagaaggagagcaaggacatcgtgaaggagctgttcaaatactga

SEQ ID NO: 26 - protein, 310 aa, Artificial Sequence
  mutant 2
MFNFIKFKFILILFLPPILFGCMAMTPNIASIRATSGPEYITSIHRDLVSLPKPENPIPVAVYKFRDQTGQYKAHPAATSPAVTQGATSILIKALEDSGWFLPVEREGLANLLQERKIVLQMRELYLTEEQKKQFEPLPPLLYAGIIFEGGIIGYDSNVTTGGIGAKYFGAGGSAEYRVDKVSIYLRAVSVKNGAVLKTVQTSKTVLSQMLSLGIFRFVRLNRLLEAEAGIAANEPVEMAVQEAIEKAVYDIIIEGVKTGIWKPKDTKEFEKWLSKYENELKEKTFASESISKLSKQKESKDIVKELFKY

SEQ ID NO: 27 - protein, 310 aa, Artificial Sequence
  mutant 3
MFNFIKFKFILILFLPPILFGCMAMTPNIASIRATSGPEYITSIHRDLVSLPKPENPIPVAVYKFRDQTGQYKPAASSLSPAVTQGATSILIKALEDSGWFLPVEREGLANLLQERKIVLQMRELYLTEEQKKQFEPLPPLLYAGIIFEGGIIGYDSNVTTGGIGAKYFGAGGSAEYRVDKVSIYLRAVSVKNGAVLKTVQTSKTVLSQMLSLGIFRFVRLNRLLEAEAGIAANEPVEMAVQEAIEKAVYDIIIEGVKTGIWKPKDTKEFEKWLSKYENELKEKTFASESISKLSKQKESKDIVKELFKY

SEQ ID NO: 28 - protein, 310 aa, Artificial Sequence
  mutant 4
MFNFIKFKFILILFLPPILFGCMAMTPNIASIRATSGPEYITSIHRDLVSLPKPENPIPVAVYKFRDQTGQYKPYPANASPAVTQGATSILIKALEDSGWFLPVEREGLANLLQERKIVLQMRELYLTEEQKKQFEPLPPLLYAGIIFEGGIIGYDSNVTTGGIGAKYFGAGGSAEYRVDKVSIYLRAVSVKNGAVLKTVQTSKTVLSQMLSLGIFRFVRLNRLLEAEAGIAANEPVEMAVQEAIEKAVYDIIIEGVKTGIWKPKDTKEFEKWLSKYENELKEKTFASESISKLSKQKESKDIVKELFKY